European Patent Specification EP 4 028 768 B1, published August 7, 2024. Title: LATERAL FLOW IMMONUASSAY DEVICE AND USES THEREOF. Applicant: DUCREST, Percevent Jérémy. The sequence listing filed with the application follows.

SEQUENCE LISTING (13 sequences)

SEQ ID NO: 1 - protein, 148 aa, Artificial sequence
  synthetic fragment 40-187 from Candida albicans Hwp1
SYDYYQEPCDDYPQQQQQQEPCDYPQQQQQEEPCDYPQQQPQEPCDYPQQPQEPCDYPQQPQEPCDYPQQPQEPCDNPPQPDVPCDNPPQPDVPCDNPPQPDVPCDNPPQPDVPCDNPPQPDQPDDNPPIPNIPTDWIPNIPTDWIPD

SEQ ID NO: 2 - protein, 160 aa, Artifical sequence
YDYYQEPCDDYPQQQQQQEPCDYPQQQQQEEPCDYPQQQPQEPCDYPQQPQEPCDYPQQPQEPCDYPQQPQEPCDNPPQPDVPCDNPPQPDVPCDNPPQPDVPCDNPPQPDVPCDNPPQPDQPDDNPPIPNIPTDWIPNIPTDWIPDIPEKPTTPATTPN

SEQ ID NO: 3 - protein, 177 aa, Artifical sequence
GQGETEEALIQKRSYDYYQEPCDDYPQQQQQQEPCDYPQQQQQEEPCDYPQQQPQEPCDYPQQPQEPCDYPQQPQEPCDYPQQPQEPCDNPPQPDVPCDNPPQPDVPCDNPPQPDVPCDNPPQPDVPCDNPPQPDQPDDNPPIPNIPTDWIPNIPTDWIPDIPEKPTTPATTPNIPA

SEQ ID NO: 4 - protein, 440 aa, Candida albicans [sequence omitted]

SEQ ID NO: 5 - protein, 308 aa, Candida albicans
MQIKFLTTLATVLTSVAAMGDLAFNLGVKNDDGTCKDVSTFEGDLDFLKSHSKIIKTYAVSDCNTLQNLGPAAEAEGFQIQLGIWPNDDAHFEAEKEALQNYLPKISVSTIKIFLVGSEALYREDLTASELASKINEIKDLVKGIKDKNGKSYSSVPVGTVDSWNVLVDGASKPAIDAADVVYSNSFSYWQKNSQANASYSLFDDVMQALQTLQTAKGSTDIEFWVGETGWPTDGSSYGDSVPSVENAADQWQKGICALRAWGINVAVYEAFDEAWKPDTSGTSSVEKHWGVWQSDKTLKYSIDCKFN

SEQ ID NO: 6 - protein, 359 aa, Candida albicans
MAPPAVLSKSGVIYGKDVKDLFDYAQEKGFAIPAINVTSSSTVVAALEAARDNKAPIILQTSQGGAAYFAGKGVDNKDQAASIAGSIAAAHYIRAIAPTYGIPVVLHTDHCAKKLLPWFDGMLKADEEFFAKTGTPLFSSHMLDLSEETDDENIATCAKYFERMAKMGQWLEMEIGITGGEEDGVNNEHVEKDALYTSPETVFAVYESLHKISPNFSIAAAFGNVHGVYKPGNVQLRPEILGDHQVYAKKQIGTDAKHPLYLVFHGGSGSTQEEFNTAIKNGVVKVNLDTDCQYAYLTGIRDYVTNKIEYLKAPVGNPEGADKPNKKYFDPRVWVREGEKTMSKRIAEALDIFHTKGQL

SEQ ID NO: 7 - protein, 238 aa, Artificial sequence
  Synthetic fragment 1-238 from Candida albicans Pgk1
MSLSNKLSVKDLDVAGKRVFIRVDFNVPLDGKTITNNQRIVAALPTIKYVEEHKPKYIVLASHLGRPNGERNDKYSLAPVATELEKLLGQKVTFLNDCVGPEVTKAVENAKDGEIFLLENLRYHIEEEGSSKDKDGKKVKADPEAVKKFRQELTSLADVYINDAFGTAHRAHSSMVGLEVPQRAAGFLMSKELEYFAKALENPERPFLAILGGAKVSDKIQLIDNLLDKVDMLIVGGG

SEQ ID NO: 8 - protein, 208 aa, Artificial sequence
  Synthetic fragment 1-208 from Candida albicans Set1
MSYNNRSGGGASGGYSRRGYHGSHRGGYRTGRSKYPEDRYLVGGMLSLNKGSHYESSDNRYIPNEIGSKSPENRSHRSSTKDGRTPSGLSTPLSSSDKVSTPISIESINGSDRNTGVNNKDSEFPKLSHHSDFTSTIPFSRSINPQKNFMVINDSHTPKTDKGIQSKKIRYNGEGVNHVSDPRIAQSNSNLQKPTKKTKKTPYKQLPQ

SEQ ID NO: 9 - protein, 751 aa, Candida albicans
MKLLPLSFSFLLFTFTFAKQLPVFDGKTYQSYSHSRNVYACRMHIHKTIKECSTTDIEDYGCMCTNKDAISTFIQCYAYFQKNSTQAIDFFVKYCDNYGNITTNIDQITDAYEDFLNNGSDTTTITNINNNNNTTNNTTSNHLDFDYSKYAYGLEASIDQFLTNWQRSFFYGMAMSSYWGFVLLFGTISNWTQYLFPGLMTDLTGPFSNWWRKNLSLPATFGTKKTQEYTFWFKYLQGYIPSRLESIINSGFCLVVIIVLSINTYYSVGNEIIFTNYVAQLRYLANRTGINSTILMPFLVLFAGRNNILQWITRWNYGVFMMFHRFIGRMIFLFVVLHAVTFSIALGVDYYPLMSFPFMIWGTISTVAGGIIMVQASLYVRRRWYEVFLGLHILLALFFMIGGWVHISYLGYEWWVFVAIGLWGIDRIVRVLRMISFGFPEADITLMSDETLKIKIPRPDYWEPIPGGHIFITFLRKDCFWQSHPFTFAPSVENSNTIVLYTKVKQGVTRKLYNYLVTCPGRRAKITVGVEGPYGECCAAGKSQTAVFIAGGNGVPGMFSEIYDLAKRSTPDSQKRLKLYWTIREYRSIHWLYEELNELKKFHNVEVTVFVTKPDSNTYINELSSRVISGKCNSTENFDGATTATTSLYEKASFDDKATIVVTNRDITSKYDPNSVKDAIIAQLSHVHFREGRPKINTIIKEEIEDAQGSICFVTCGHPAMVDDIRAEVVGTIGKYKEKRIDYYEQLIGWA

SEQ ID NO: 10 - protein, 20 aa, Artificial sequence
  Synthetic
QEPCDYPQQPQEPCDYPQQP

SEQ ID NO: 11 - protein, 14 aa, Artificial sequence
  Synthetic
DSRGNPTVEVDFTT

SEQ ID NO: 12 - protein, 14 aa, Artificial sequence
  Synthetic
YGKDVKDLFDYAQE

SEQ ID NO: 13 - protein, 14 aa, Artificial sequence
  Synthetic
VPLDGKTITNNQRI